European Patent Application EP 4 681 731 A1, published January 21, 2026. Title: USE OF ANTI-OX40 ANTIBODY IN TREATMENT OF INFLAMMATORY OR IMMUNE DISEASES. Applicant: Bio-Thera Solutions, Ltd. Application EP. The sequence listing filed with the application follows.

SEQUENCE LISTING (12 sequences)

SEQ ID NO: 1 - protein, 5 aa, synthetic construct
SYGMH

SEQ ID NO: 2 - protein, 17 aa, synthetic construct
VIWEDGSNQYYADSVKG

SEQ ID NO: 3 - protein, 13 aa, synthetic construct
DNQDTSPDVGIDY

SEQ ID NO: 4 - protein, 11 aa, synthetic construct
RASQNISPFLN

SEQ ID NO: 5 - protein, 7 aa, synthetic construct
AAVGLQS

SEQ ID NO: 6 - protein, 9 aa, synthetic construct
QQYTDYPLT

SEQ ID NO: 7 - protein, 122 aa, synthetic construct
QVQLVESGGGVVQPGESLRLSCAASGFTFSSYGMHWVRQAPGKGLEWVAVIWEDGSNQYYADSVKGRFTISRDNSKNTLYLQMNSLRAEDTAVYYCAKDNQDTSPDVGIDYWGQGTLVTVSS

SEQ ID NO: 8 - protein, 107 aa, synthetic construct
DIQMTQSPSSLSASVGDRVTITCRASQNISPFLNWYQQKPGKAPKLLIYAAVGLQSGVPSRFSGSGSGTDFTLTISSLQPEDFATYYCQQYTDYPLTFGGGTKVEIK

SEQ ID NO: 9 - protein, 452 aa, synthetic construct
QVQLVESGGGVVQPGESLRLSCAASGFTFSSYGMHWVRQAPGKGLEWVAVIWEDGSNQYYADSVKGRFTISRDNSKNTLYLQMNSLRAEDTAVYYCAKDNQDTSPDVGIDYWGQGTLVTVSSASTKGPSVFPLAPSSKSTSGGTAALGCLVKDYFPEPVTVSWNSGALTSGVHTFPAVLQSSGLYSLSSVVTVPSSSLGTQTYICNVNHKPSNTKVDKKVEPKSCDKTHTCPPCPAPELLGGPSVFLFPPKPKDTLMISRTPEVTCVVVDVSHEDPEVKFNWYVDGVEVHNAKTKPREEQYNSTYRVVSVLTVLHQDWLNGKEYKCKVSNKALPAPIEKTISKAKGQPREPQVYTLPPSRDELTKNQVSLTCLVKGFYPSDIAVEWESNGQPENNYKTTPPVLDSDGSFFLYSKLTVDKSRWQQGNVFSCSVMHEALHNHYTQKSLSLSPGK

SEQ ID NO: 10 - protein, 214 aa, synthetic construct
DIQMTQSPSSLSASVGDRVTITCRASQNISPFLNWYQQKPGKAPKLLIYAAVGLQSGVPSRFSGSGSGTDFTLTISSLQPEDFATYYCQQYTDYPLTFGGGTKVEIKRTVAAPSVFIFPPSDEQLKSGTASVVCLLNNFYPREAKVQWKVDNALQSGNSQESVTEQDSKDSTYSLSSTLTLSKADYEKHKVYACEVTHQGLSSPVTKSFNRGEC

SEQ ID NO: 11 - protein, 447 aa, synthetic construct
QITLKESGPTLVKPKQTLTLTCTFSGFSLSTSGMGVGWIRQPPGKALEWLAVIYWDDHQLYSPSLKSRLTITKDTSKNQVVLTMTNMDPVDTATYYCAHRRGAFQHWGQGTLVTVSSASTKGPSVFPLAPSSKSTSGGTAALGCLVKDYFPEPVTVSWNSGALTSGVHTFPAVLQSSGLYSLSSVVTVPSSSLGTQTYICNVNHKPSNTKVDKKVEPKSCDKTHTCPPCPAPELLGGPSVFLFPPKPKDTLMISRTPEVTCVVVDVSHEDPEVKFNWYVDGVEVHNAKTKPREEQYNSTYRVVSVLTVLHQDWLNGKEYKCKVSNKALPAPIEKTISKAKGQPREPQVYTLPPSRDELTKNQVSLTCLVKGFYPSDIAVEWESNGQPENNYKTTPPVLDSDGSFFLYSKLTVDKSRWQQGNVFSCSVMHEALHNHYTQKSLSLSPGK

SEQ ID NO: 12 - protein, 214 aa, synthetic construct
EIVLTQSPGTLSLSPGERATLSCRASQSVSSSYLAWYQQKPGQAPRLLIYGASSRATGIPDRFSGSGSGTDFTLTISRLEPEDFAVYYCQQYDSSLTFGGGTKVEIKRTVAAPSVFIFPPSDEQLKSGTASVVCLLNNFYPREAKVQWKVDNALQSGNSQESVTEQDSKDSTYSLSSTLTLSKADYEKHKVYACEVTHQGLSSPVTKSFNRGEC